European Patent Specification EP 3 608 336 B1, published October 2, 2024. Title: pan-ELR+ CXC Chemokine Antibodies. Applicant: Eli Lilly and Company. The sequence listing filed with the application follows.

SEQUENCE LISTING (27 sequences)

SEQ ID NO: 1 - protein, 452 aa, Artificial Sequence
  synthetic construct
QVQLVQSGAEVKKPGASVKVSCKASGYEFTSYWIHWVRQAPGQGLEWMGNISPNSGSANYNEKFKSRVTMTRDTSTSTVYMELSSLRSEDTAVYYCAREGPYSYYPSREYYGSDLWGQGTLVTVSSASTKGPSVFPLAPCSRSTSESTAALGCLVKDYFPEPVTVSWNSGALTSGVHTFPAVLQSSGLYSLSSVVTVPSSSLGTKTYTCNVDHKPSNTKVDKRVESKYGPPCPPCPAPEFLGGPSVFLFPPKPKDTLMISRTPEVTCVVVDVSQEDPEVQFNWYVDGVEVHNAKTKPREEQFNSTYRVVSVLTVLHQDWLNGKEYKCKVSNKGLPSSIEKTISKAKGQPREPQVYTLPPSQEEMTKNQVSLTCLVKGFYPSDIAVEWESNGQPENNYKTTPPVLDSDGSFFLYSRLTVDKSRWQEGNVFSCSVMHEALHNHYTQKSLSLSLG

SEQ ID NO: 2 - protein, 126 aa, Artificial Sequence
  synthetic construct
QVQLVQSGAEVKKPGASVKVSCKASGYEFTSYWIHWVRQAPGQGLEWMGNISPNSGSANYNEKFKSRVTMTRDTSTSTVYMELSSLRSEDTAVYYCAREGPYSYYPSREYYGSDLWGQGTLVTVSS

SEQ ID NO: 3 - protein, 214 aa, Artificial Sequence
  synthetic construct
EIVLTQSPATLSLSPGERATLSCRASQSISNNLHWYQQKPGQAPRLLIYYTSRSVSGIPARFSGSGSGTDFTLTISSLEPEDFAVYYCGQNNEWPEVFGGGTKVEIKRTVAAPSVFIFPPSDEQLKSGTASVVCLLNNFYPREAKVQWKVDNALQSGNSQESVTEQDSKDSTYSLSSTLTLSKADYEKHKVYACEVTHQGLSSPVTKSFNRGEC

SEQ ID NO: 4 - protein, 107 aa, Artificial Sequence
  synthetic construct
EIVLTQSPATLSLSPGERATLSCRASQSISNNLHWYQQKPGQAPRLLIYYTSRSVSGIPARFSGSGSGTDFTLTISSLEPEDFAVYYCGQNNEWPEVFGGGTKVEIK

SEQ ID NO: 5 - DNA, 1356 bp, Artificial Sequence
  synthetic construct
caggtgcagctggtgcagtctggtgctgaagtgaagaagcctggggcctcagtgaaggtgtcctgcaaggcatctggctacgagttcaccagctactggattcactgggtgcgacaggcccctggacaagggcttgagtggatgggaaatatttctcctaatagtggtagtgctaactacaatgagaagttcaagagcagagtcaccatgaccagggacacgtccacgagcacagtctacatggagctgagcagcctgagatctgaggacacggccgtgtattactgtgcgagagagggcccttacagttattatccgagtagggagtactatggctctgacctctgggggcaagggaccctagtcacagtctcctcagcctccaccaagggcccatcggtcttcccgctagcgccctgctccaggagcacctccgagagcacagccgccctgggctgcctggtcaaggactacttccccgaaccggtgacggtgtcgtggaactcaggcgccctgaccagcggcgtgcacaccttcccggctgtcctacagtcctcaggactctactccctcagcagcgtggtgaccgtgccctccagcagcttgggcacgaagacctacacctgcaacgtagatcacaagcccagcaacaccaaggtggacaagagagttgagtccaaatatggtcccccatgcccaccctgcccagcacctgagttcctggggggaccatcagtcttcctgttccccccaaaacccaaggacactctcatgatctcccggacccctgaggtcacgtgcgtggtggtggacgtgagccaggaagaccccgaggtccagttcaactggtacgtggatggcgtggaggtgcataatgccaagacaaagccgcgggaggagcagttcaacagcacgtaccgtgtggtcagcgtcctcaccgtcctgcaccaggactggctgaacggcaaggagtacaagtgcaaggtctccaacaaaggcctcccgtcctccatcgagaaaaccatctccaaagccaaagggcagccccgagagccacaggtgtacaccctgcccccatcccaggaggagatgaccaagaaccaggtcagcctgacctgcctggtcaaaggcttctaccccagcgacatcgccgtggagtgggaaagcaatgggcagccggagaacaactacaagaccacgcctcccgtgctggactccgacggctccttcttcctctacagcaggctaaccgtggacaagagcaggtggcaggaggggaatgtcttctcatgctccgtgatgcatgaggctctgcacaaccactacacacagaagagcctctccctgtctctgggt

SEQ ID NO: 6 - DNA, 642 bp, Artificial Sequence
  synthetic construct
gaaattgtgttgacacagtctccagccaccctgtctttgtctccaggggaaagagccaccctctcctgcagggccagtcaaagtatcagcaataacctacactggtaccaacagaaacctggccaggctcccaggctcctcatctattatacttcccggtccgtctctggcatcccagccaggttcagtggcagtgggtctgggacagacttcactctcaccatcagcagcctagagcctgaagattttgcagtttattactgtggacagaataacgagtggcctgaggtgttcggcggagggaccaaggtggagatcaaacgaactgtggctgcaccatctgtcttcatcttcccgccatctgatgagcagttgaaatctggaactgcctctgttgtgtgcctgctgaataacttctatcccagagaggccaaagtacagtggaaggtggataacgccctccaatcgggtaactcccaggagagtgtcacagagcaggacagcaaggacagcacctacagcctcagcagcaccctgacgctgagcaaagcagactacgagaaacacaaagtctacgcctgcgaagtcacccatcagggcctgagctcgcccgtcacaaagagcttcaacaggggagagtgc

SEQ ID NO: 7 - protein, 11 aa, Artificial Sequence
  synthetic construct
RASQSISNNLH

SEQ ID NO: 8 - protein, 7 aa, Artificial Sequence
  synthetic construct
YTSRSVS

SEQ ID NO: 9 - protein, 9 aa, Artificial Sequence
  synthetic construct
GQNNEWPEV

SEQ ID NO: 10 - protein, 10 aa, Artificial Sequence
  synthetic construct
GYEFTSYWIH

SEQ ID NO: 11 - protein, 17 aa, Artificial Sequence
  synthetic construct
NISPNSGSANYNEKFKS

SEQ ID NO: 12 - protein, 17 aa, Artificial Sequence
  synthetic construct
EGPYSYYPSREYYGSDL

SEQ ID NO: 13 - protein, 452 aa, Artificial Sequence
  synthetic construct
QVQLVQSGAEVKKPGASVKVSCKASGYEFTSYWIHWVRQAPGQGLEWMGNISPNSGSANYNEKFKSRVTMTRDTSTSTVYMELSSLRSEDTAVYYCAREGPYSYYPSRQYYGSDLWGQGTLVTVSSASTKGPSVFPLAPCSRSTSESTAALGCLVKDYFPEPVTVSWNSGALTSGVHTFPAVLQSSGLYSLSSVVTVPSSSLGTKTYTCNVDHKPSNTKVDKRVESKYGPPCPPCPAPEFLGGPSVFLFPPKPKDTLMISRTPEVTCVVVDVSQEDPEVQFNWYVDGVEVHNAKTKPREEQFNSTYRVVSVLTVLHQDWLNGKEYKCKVSNKGLPSSIEKTISKAKGQPREPQVYTLPPSQEEMTKNQVSLTCLVKGFYPSDIAVEWESNGQPENNYKTTPPVLDSDGSFFLYSRLTVDKSRWQEGNVFSCSVMHEALHNHYTQKSLSLSLG

SEQ ID NO: 14 - protein, 126 aa, Artificial Sequence
  synthetic construct
QVQLVQSGAEVKKPGASVKVSCKASGYEFTSYWIHWVRQAPGQGLEWMGNISPNSGSANYNEKFKSRVTMTRDTSTSTVYMELSSLRSEDTAVYYCAREGPYSYYPSRQYYGSDLWGQGTLVTVSS

SEQ ID NO: 15 - protein, 214 aa, Artificial Sequence; identical to SEQ ID NO: 3
  synthetic construct

SEQ ID NO: 16 - protein, 107 aa, Artificial Sequence; identical to SEQ ID NO: 4
  synthetic construct

SEQ ID NO: 17 - DNA, 1356 bp, Artificial Sequence
  synthetic construct
caggtgcagctggtgcagtctggtgctgaagtgaagaagcctggggcctcagtgaaggtgtcctgcaaggcatctggctacgagttcaccagctactggattcactgggtgcgacaggcccctggacaagggcttgagtggatgggaaatatttctcctaatagtggtagtgctaactacaatgagaagttcaagagcagagtcaccatgaccagggacacgtccacgagcacagtctacatggagctgagcagcctgagatctgaggacacggccgtgtattactgtgcgagagagggcccttacagttattatccgagtaggcagtactatggctctgacctctgggggcaagggaccctagtcacagtctcctcagcctccaccaagggcccatcggtcttcccgctagcgccctgctccaggagcacctccgagagcacagccgccctgggctgcctggtcaaggactacttccccgaaccggtgacggtgtcgtggaactcaggcgccctgaccagcggcgtgcacaccttcccggctgtcctacagtcctcaggactctactccctcagcagcgtggtgaccgtgccctccagcagcttgggcacgaagacctacacctgcaacgtagatcacaagcccagcaacaccaaggtggacaagagagttgagtccaaatatggtcccccatgcccaccctgcccagcacctgagttcctggggggaccatcagtcttcctgttccccccaaaacccaaggacactctcatgatctcccggacccctgaggtcacgtgcgtggtggtggacgtgagccaggaagaccccgaggtccagttcaactggtacgtggatggcgtggaggtgcataatgccaagacaaagccgcgggaggagcagttcaacagcacgtaccgtgtggtcagcgtcctcaccgtcctgcaccaggactggctgaacggcaaggagtacaagtgcaaggtctccaacaaaggcctcccgtcctccatcgagaaaaccatctccaaagccaaagggcagccccgagagccacaggtgtacaccctgcccccatcccaggaggagatgaccaagaaccaggtcagcctgacctgcctggtcaaaggcttctaccccagcgacatcgccgtggagtgggaaagcaatgggcagccggagaacaactacaagaccacgcctcccgtgctggactccgacggctccttcttcctctacagcaggctaaccgtggacaagagcaggtggcaggaggggaatgtcttctcatgctccgtgatgcatgaggctctgcacaaccactacacacagaagagcctctccctgtctctgggt

SEQ ID NO: 18 - DNA, 642 bp, Artificial Sequence; identical to SEQ ID NO: 6
  synthetic construct

SEQ ID NO: 19 - protein, 17 aa, Artificial Sequence
  synthetic construct
EGPYSYYPSRQYYGSDL

SEQ ID NO: 20 - protein, 17 aa, Artificial Sequence
  synthetic construct
  MISC_FEATURE (11)..(11): Xaa position 11 is Glu or Gln
EGPYSYYPSRXYYGSDL

SEQ ID NO: 21 - protein, 73 aa, Homo sapiens
ASVATELRCQCLQTLQGIHPKNIQSVNVKSPGPHCAQTEVIATLKNGRKACLNPASPIVKKIIEKMLNSDKSN

SEQ ID NO: 22 - protein, 73 aa, Homo sapiens
APLATELRCQCLQTLQGIHLKNIQSVKVKSPGPHCAQTEVIATLKNGQKACLNPASPMVKKIIEKMLKNGKSN

SEQ ID NO: 23 - protein, 73 aa, Homo sapiens
ASVVTELRCQCLQTLQGIHLKNIQSVNVRSPGPHCAQTEVIATLKNGKKACLNPASPMVQKIIEKILNKGSTN

SEQ ID NO: 24 - protein, 74 aa, Homo sapiens
AAVLRELRCVCLQTTQGVHPKMISNLQVFAIGPQCSKVEVVASLKNGKEICLDPEAPFLKKVIQKILDGGNKEN

SEQ ID NO: 25 - protein, 75 aa, Homo sapiens
VSAVLTELRCTCLRVTLRVNPKTIGKLQVFPAGPQCSKVEVVASLKNGKQVCLDPEAPFLKKVIQKILDSGNKKN

SEQ ID NO: 26 - protein, 70 aa, Homo sapiens
AELRCMCIKTTSGIHPKNIQSLEVIGKGTHCNQVEVIATLKDGRKICLDPDAPRIKKIVQKKLAGDESAD

SEQ ID NO: 27 - protein, 72 aa, Homo sapiens
SAKELRCQCIKTYSKPFHPKFIKELRVIESGPHCANTEIIVKLSDGRELCLDPKENWVQRVVEKFLKRAENS